European Patent Specification EP 3 856 228 B1, published March 8, 2023. Title: METHODS AND PHARMACEUTICAL COMPOSITION REDUCING SKIN INFLAMMATION. Applicant: Inserm. The sequence listing filed with the application follows.

SEQUENCE LISTING (2 sequences)

SEQ ID NO: 1 - protein, 140 aa, Homo sapiens
MRSPRMRVCAKSVLLSHWLFLAYVLMVCCKLMSASSQHLRGHAGHHQIKQGTCEVVAVHRCCNKNRIEERSQTVKCSCFPGQVAGTTRAQPSCVEASIVIQKWWCHMNPCLEGEDCKVLPDYSGWSCSSGNKVKTTKVTR

SEQ ID NO: 2 - DNA, 2294 bp, Homo sapiens
aatcagcgcgttccgcggcgggcccggcccctcctggtcagcgcgctagctgggctcggctccgcactgctagctgcgcgccgccctggacggggcgcaccgactgcgcgcgcggctgcgggcaaacatcgggagtcctgcctcagctgccgcttctccagcagcagcttcaggcttctcccgcaggagcttcgggcttctcctggtagagacgtgggaacttttcttctcctggcgaggctgcagaggtgatgggccgctcccggggctcccgcggggaggcggcacggtgagcgtcctcgggctccggtgcggcgatcagtacctagttccggacgcgccggtccgacttggatgccggctctagtcgagtcttctgagctacgataattttttggaacggcagaaatgattggttctagcaacagatgggaatttggagtcactctgaaatatatcctggaataagtgtgtttgactagaaccacatcttatgaggtccccaaggatgagagtctgtgctaagtcagtgttgctgtcgcactggctctttctagcctacgtgttaatggtgtgctgtaagctgatgtccgcctcaagccagcacctccggggacatgcaggtcaccaccaaatcaagcaagggacctgtgaggtggtcgccgtgcacaggtgctgcaataagaaccgcatagaagagcggtcacaaacggtcaagtgctcttgcttcccgggacaggtggcgggcacaactcgggctcaaccttcttgtgttgaagcttccattgtgattcagaaatggtggtgtcacatgaatccgtgtttggaaggagaggattgtaaagtgctgccagattactcaggttggtcctgtagcagtggcaataaagtcaaaactacgaaggtaacgcggtagcgaagagagaggtgtgcttcaatcctggaggggcagcaggaggcggagctcttttgcttggattcccatcatggcccctttgcagaaaattgtctaggatttcagcaacttcatatttgtatatgtgagctgtgagaggtggcattcacttaactggcccagccctctctgcttcgtgattttatttcattgaattataaccacaagccaccacccatttgacatcctctctggattcccaaggagcatacctccaaaatccgagaagagcaaatcagagtcttcaaaatggatcaccactaagggcatgttcattcttcactttctttctgcttttacaaaagaacttggatgtatgttccaaagggtcctcattctgttcctcttttgaacttttccttttgtccttgtattaaagtggttttaaaggggtctaaaaagattttggcaaaacatatttgcagatgtagattagctggtgaagaaaattactgctagagatcaactgattaactggtaaagaacgtttattttataacccttgaagaatagaaggacatagttggattattgtgtgtgcattgtatttttacttctattttttttttgctttccattttccagttagcagagataaaatgagagcgttttaacttcaatgtaccattttactgagtgctaaggaagcatatcaattccaatattttataaccaaagctctatcagaacatatttataaaacttgttggaatttttacggcttttgtgtagtcatgtaggtaaatcatttaaaatataaaacaatctcaatttagatcaagggttatttcttagatcaaatttatgccaattatatgaaaagattttaactccgagacaggagtctttcagtgctgaatttttagactgtaaatgagttcttcttaacttagctgtttccctacttctgtgacttctgtgttagccatcttatttctttaaaatctgagtcctgattggcttaatgattttgcagcagacatgtctccacatattctcaaatgctgtcatgcggaaacgtatgaaacagatgaagaatgactgacccagattttagatgtataatgttgttaaagtacatactactgtaaaaatatgggatgaattttatatattaagaaatgccaaaaacatagtttctgcaccaagttaattatccctgtcctttcacatttatagggggaaaataaatactttaatgttgtttatagcctaacagttatttgattttattcttgcagagggaatggaaaggaatggaaagatttgttggcgtaatttttgaatatttgttatgatcatatgaataagtaaaaaaattcatcctgctgatggcata